European Patent Application EP 4 338 755 A1, published March 20, 2024. Title: USING MINIVECTORS TO TREAT IDIOPATHIC PULMONARY FIBROSIS. Applicant: BAYLOR COLLEGE OF MEDICINE. Application US US 17/930,298, filed September 7, 2022. The sequence listing filed with the application follows.

SEQUENCE LISTING (89 sequences)

SEQ ID NO: 1 - DNA, 19 bp, synthetic construct
  misc_feature 1..19: note = Synthetic: V2LHS_150470
  source 1..19: mol_type = other DNA
tactgtacactaacttggc

SEQ ID NO: 2 - DNA, 19 bp, synthetic construct
  misc_feature 1..19: note = Synthetic: V2LHS_150474
  source 1..19: mol_type = other DNA
taaatcttggtccattggc

SEQ ID NO: 3 - DNA, 19 bp, synthetic construct
  misc_feature 1..19: note = Synthetic: V3LHS_400950
  source 1..19: mol_type = other DNA
aacattttcttacatgtca

SEQ ID NO: 4 - DNA, 19 bp, synthetic construct
  misc_feature 1..19: note = Synthetic: V3LHS_400949
  source 1..19: mol_type = other DNA
aacacataaacaatttccc

SEQ ID NO: 5 - DNA, 19 bp, synthetic construct
  misc_feature 1..19: note = Synthetic: V2LHS_88502
  source 1..19: mol_type = other DNA
tacctaaggccatgaactt

SEQ ID NO: 6 - DNA, 19 bp, synthetic construct
  misc_feature 1..19: note = Synthetic: V3LHS_641819
  source 1..19: mol_type = other DNA
attgctgcaggtcgttggt

SEQ ID NO: 7 - DNA, 19 bp, synthetic construct
  misc_feature 1..19: note = Synthetic: V3LHS_641817
  source 1..19: mol_type = other DNA
tgcatgtctccttgactct

SEQ ID NO: 8 - DNA, 19 bp, synthetic construct
  misc_feature 1..19: note = Synthetic: V3LHS_641818
  source 1..19: mol_type = other DNA
aagctgataattcaactca

SEQ ID NO: 9 - DNA, 19 bp, synthetic construct
  misc_feature 1..19: note = Synthetic: V3LHS_645974
  source 1..19: mol_type = other DNA
atctttctgcagcttccgt

SEQ ID NO: 10 - DNA, 19 bp, synthetic construct
  misc_feature 1..19: note = Synthetic: V3LHS_376018
  source 1..19: mol_type = other DNA
tagtagtgaactggacgcc

SEQ ID NO: 11 - DNA, 19 bp, synthetic construct
  misc_feature 1..19: note = Synthetic: V3LHS_376016
  source 1..19: mol_type = other DNA
atagttgaaatcaaagtca

SEQ ID NO: 12 - DNA, 19 bp, synthetic construct
  misc_feature 1..19: note = Synthetic: V2LHS_153578
  source 1..19: mol_type = other DNA
tagcatatgtcagagaggc

SEQ ID NO: 13 - DNA, 19 bp, synthetic construct
  misc_feature 1..19: note = Synthetic: V3LHS_369098
  source 1..19: mol_type = other DNA
atctgtggagagccatcct

SEQ ID NO: 14 - DNA, 19 bp, synthetic construct
  misc_feature 1..19: note = Synthetic: V3LHS_369101
  source 1..19: mol_type = other DNA
agctctccagtggtctcct

SEQ ID NO: 15 - DNA, 19 bp, synthetic construct
  misc_feature 1..19: note = Synthetic: V2LHS_111877
  source 1..19: mol_type = other DNA
tagttggtgtccagggctc

SEQ ID NO: 16 - DNA, 19 bp, synthetic construct
  misc_feature 1..19: note = Synthetic: V3LHS_356823
  source 1..19: mol_type = other DNA
tgatgtccacttgcagtgt

SEQ ID NO: 17 - DNA, 19 bp, synthetic construct
  misc_feature 1..19: note = Synthetic: V3LHS_356824
  source 1..19: mol_type = other DNA
atgctgtgtgtactctgct

SEQ ID NO: 18 - DNA, 19 bp, synthetic construct
  misc_feature 1..19: note = Synthetic: V3LHS_356827
  source 1..19: mol_type = other DNA
ttctggtacagctccacgt

SEQ ID NO: 19 - DNA, 19 bp, synthetic construct
  misc_feature 1..19: note = Synthetic: V3LHS_356825
  source 1..19: mol_type = other DNA
actctgcttgaacttgtca

SEQ ID NO: 20 - DNA, 19 bp, synthetic construct
  misc_feature 1..19: note = Synthetic: V2LHS_216496
  source 1..19: mol_type = other DNA
tagtagacaatagagcacc

SEQ ID NO: 21 - DNA, 19 bp, synthetic construct
  misc_feature 1..19: note = Synthetic: V2LHS_197114
  source 1..19: mol_type = other DNA
agacaatagagcaccagtg

SEQ ID NO: 22 - DNA, 19 bp, synthetic construct
  misc_feature 1..19: note = Synthetic: V2LHS_196344
  source 1..19: mol_type = other DNA
taagatacagatgaaatag

SEQ ID NO: 23 - DNA, 19 bp, synthetic construct
  misc_feature 1..19: note = Synthetic: V3LHS_317711
  source 1..19: mol_type = other DNA
tcctcataagcaaccgcct

SEQ ID NO: 24 - DNA, 19 bp, synthetic construct
  misc_feature 1..19: note = Synthetic: V3LHS_317709
  source 1..19: mol_type = other DNA
aactgagcaaattcttggt

SEQ ID NO: 25 - DNA, 19 bp, synthetic construct
  misc_feature 1..19: note = Synthetic: V3LHS_317710
  source 1..19: mol_type = other DNA
tcgctgtgtcttggaacca

SEQ ID NO: 26 - DNA, 19 bp, synthetic construct
  misc_feature 1..19: note = Synthetic: V2LHS_169791
  source 1..19: mol_type = other DNA
tctgttaatacaggtaaag

SEQ ID NO: 27 - DNA, 19 bp, synthetic construct
  misc_feature 1..19: note = Synthetic: V2LHS_169788
  source 1..19: mol_type = other DNA
tttaggaaatgatgcatag

SEQ ID NO: 28 - DNA, 19 bp, synthetic construct
  misc_feature 1..19: note = Synthetic: V2LHS_169787
  source 1..19: mol_type = other DNA
tgggcttaaatactacagc

SEQ ID NO: 29 - DNA, 19 bp, synthetic construct
  misc_feature 1..19: note = Synthetic: V2LHS_169786
  source 1..19: mol_type = other DNA
aggttcaggaatgtaacac

SEQ ID NO: 30 - DNA, 19 bp, synthetic construct
  misc_feature 1..19: note = Synthetic: V2LHS_169790
  source 1..19: mol_type = other DNA
aaagaatttgggttctgtc

SEQ ID NO: 31 - DNA, 19 bp, synthetic construct
  misc_feature 1..19: note = Synthetic: V3LHS_340444
  source 1..19: mol_type = other DNA
aaatgaccgtcctggtctt

SEQ ID NO: 32 - DNA, 19 bp, synthetic construct
  misc_feature 1..19: note = Synthetic: V3LHS_340445
  source 1..19: mol_type = other DNA
tgacactgctcgtgttgca

SEQ ID NO: 33 - DNA, 19 bp, synthetic construct
  misc_feature 1..19: note = Synthetic: V2LHS_171350
  source 1..19: mol_type = other DNA
tattaaggtagagaggtgg

SEQ ID NO: 34 - DNA, 19 bp, synthetic construct
  misc_feature 1..19: note = Synthetic: V2LHS_221582
  source 1..19: mol_type = other DNA
tttgtttcaaattggaatg

SEQ ID NO: 35 - DNA, 19 bp, synthetic construct
  misc_feature 1..19: note = Synthetic: V3LHS_374708
  source 1..19: mol_type = other DNA
tcatttctaaattctccca

SEQ ID NO: 36 - DNA, 19 bp, synthetic construct
  misc_feature 1..19: note = Synthetic: V3LHS_374709
  source 1..19: mol_type = other DNA
tactttgaatcttgttgct

SEQ ID NO: 37 - DNA, 19 bp, synthetic construct
  misc_feature 1..19: note = Synthetic: V3LHS_374710
  source 1..19: mol_type = other DNA
agactacttggaaaatgct

SEQ ID NO: 38 - DNA, 19 bp, synthetic construct
  misc_feature 1..19: note = Synthetic: V3LHS_374707
  source 1..19: mol_type = other DNA
tctttactagctcattcct

SEQ ID NO: 39 - DNA, 19 bp, synthetic construct
  misc_feature 1..19: note = Synthetic: V2LHS_11941
  source 1..19: mol_type = other DNA
tatgtactgacctaaatag

SEQ ID NO: 40 - DNA, 19 bp, synthetic construct
  misc_feature 1..19: note = Synthetic: V2LHS_151660
  source 1..19: mol_type = other DNA
atctgaataccaatccttc

SEQ ID NO: 41 - DNA, 19 bp, synthetic construct
  misc_feature 1..19: note = Synthetic: V3LHS_356802
  source 1..19: mol_type = other DNA
tgaacactgagcagaggtg

SEQ ID NO: 42 - DNA, 19 bp, synthetic construct
  misc_feature 1..19: note = Synthetic: V3LHS_356797
  source 1..19: mol_type = other DNA
aacagtgaacatttcacct

SEQ ID NO: 43 - DNA, 106 bp, synthetic construct
  misc_feature 1..106: note = Synthetic: l-attL
  source 1..106: mol_type = other DNA
tccgttgaagcctgcttttttatactaagttggcattataaaaaagcattgcttatcaatttgttgcaacgaacaggtcactatcagtcaaaataaaatcattatt

SEQ ID NO: 44 - DNA, 183 bp, synthetic construct
  misc_feature 1..183: note = Synthetic: l-attR
  source 1..183: mol_type = other DNA
agatgcctcagctctgttacaggtcactaataccatctaagtagttgattcatagtgactgcatatgttgtgttttacagtattatgtagtctgttttttatgcaaaatctaatttaatatattgatatttatatcattttacgtttctcgttcagcttttttatactaacttgagcgaaacg

SEQ ID NO: 45 - DNA, 41 bp, synthetic construct
  misc_feature 1..41: note = Synthetic: l-attB
  source 1..41: mol_type = other DNA
tccgttgaagcctgcttttttatactaacttgagcgaaacg

SEQ ID NO: 46 - DNA, 248 bp, synthetic construct
  misc_feature 1..248: note = Synthetic: l-attP
  source 1..248: mol_type = other DNA
agatgcctcagctctgttacaggtcactaataccatctaagtagttgattcatagtgactgcatatgttgtgttttacagtattatgtagtctgttttttatgcaaaatctaatttaatatattgatatttatatcattttacgtttctcgttcagcttttttatactaagttggcattataaaaaagcattgcttatcaatttgttgcaacgaacaggtcactatcagtcaaaataaaatcattatt

SEQ ID NO: 47 - DNA, 34 bp, synthetic construct
  misc_feature 1..34: note = Synthetic: loxP
  source 1..34: mol_type = other DNA
ataacttcgtatagcatacattatacgaagttat

SEQ ID NO: 48 - DNA, 130 bp, synthetic construct
  misc_feature 1..130: note = Synthetic: gd-res
  source 1..130: mol_type = other DNA
attttgcaaccgtccgaaatattataaattatcgcacacataaaaacagtgctgttaatgtgtctattaaatcgattttttgttataacagacactgcttgtccgatatttgatttaggatacattttta

SEQ ID NO: 49 - DNA, 34 bp, synthetic construct
  misc_feature 1..34: note = Synthetic: FRT
  source 1..34: mol_type = other DNA
gaagttcctattctctagaaagtataggaacttc

SEQ ID NO: 50 - DNA, 26 bp, synthetic construct
  misc_feature 1..26: note = Synthetic: hixL
  source 1..26: mol_type = other DNA
ttcttgaaaaccaaggtttttgataa

SEQ ID NO: 51 - DNA, 26 bp, synthetic construct
  misc_feature 1..26: note = Synthetic: hixR
  source 1..26: mol_type = other DNA
ttttccttttggaaggtttttgataa

SEQ ID NO: 52 - DNA, 121 bp, synthetic construct
  misc_feature 1..121: note = Synthetic: Tn3 res
  source 1..121: mol_type = other DNA
caaccgttcgaaatattataaattatcagacatagtaaaacggcttcgtttgagtgtccattaaatcgtcattttggcataatagacacatcgtgtctgatattcgatttaaggtacattt

SEQ ID NO: 53 - DNA, 126 bp, synthetic construct
  misc_feature 1..126: note = Synthetic: Tn21 res
  source 1..126: mol_type = other DNA
gccgccgtcaggttgaggcataccctaacctgatgtcagatgccatgtgtaaattgcgtcaggataggattgaattttgaatttattgacatatctcgttgaaggtcatagagtcttccctgacat

SEQ ID NO: 54 - DNA, 30 bp, synthetic construct
  misc_feature 1..30: note = Synthetic: cer
  source 1..30: mol_type = other DNA
ggtgcgtacaattaagggattatggtaaat

SEQ ID NO: 55 - DNA, 28 bp, synthetic construct
  misc_feature 1..28: note = Synthetic: psi
  source 1..28: mol_type = other DNA
ggtgcgcgcaagatccattatgttaaac

SEQ ID NO: 56 - DNA, 584 bp, unidentified
  misc_feature 1..584: note = Promoter from the human cytomegalovirus (CMV)
  source 1..584: mol_type = unassigned DNA
gacattgattattgactagttattaatagtaatcaattacggggtcattagttcatagcccatatatggagttccgcgttacataacttacggtaaatggcccgcctggctgaccgcccaacgacccccgcccattgacgtcaataatgacgtatgttcccatagtaacgccaatagggactttccattgacgtcaatgggtggagtatttacggtaaactgcccacttggcagtacatcaagtgtatcatatgccaagtacgccccctattgacgtcaatgacggtaaatggcccgcctggcattatgcccagtacatgaccttatgggactttcctacttggcagtacatctacgtattagtcatcgctattaccatggtgatgcggttttggcagtacatcaatgggcgtggatagcggtttgactcacggggatttccaagtctccaccccattgacgtcaatgggagtttgttttggcaccaaaatcaacgggactttccaaaatgtcgtaacaactccgccccattgacgcaaatgggcggtaggcgtgtacggtgggaggtctatataagcagagct

SEQ ID NO: 57 - DNA, 100 bp, unidentified
  misc_feature 1..100: note = mini-CMV
  source 1..100: mol_type = unassigned DNA
ccaaaatcaacgggactttccaaaatgtcgtaacaactccgccccattgacgcaaatgggcggtaggcgtgtacggtgggaggtctatataagcagagct

SEQ ID NO: 58 - DNA, 262 bp, Rous sarcoma virus
  misc_feature 1..262: note = Long terminal repeat (LTR) of the rous sarcoma virus (RSV)
  source 1..262: mol_type = genomic DNA
ggtgcacaccaatgtggtgaatggtcaaatggcgtttattgtatcgagctaggcacttaaatacaatatctctgcaatgcggaattcagtggttcgtccaatccatgtcagacccgtctgttgccttcctaataaggcacgatcgtaccaccttacttccaccaatcggcatgcacggtgctttttctctccttgtaaggcatgttgctaactcatcgttaccatgttgcaagactacaagagtattgcataagactacatt

SEQ ID NO: 59 - DNA, 584 bp, synthetic construct
  misc_feature 1..584: note = Synthetic: CAG
  source 1..584: mol_type = other DNA
gcgttacataacttacggtaaatggcccgcctggctgaccgcccaacgacccccgcccattgacgtcaataatgacgtatgttcccatagtaacgccaatagggactttccattgacgtcaatgggtggagtatttacggtaaactgcccacttggcagtacatcaagtgtatcatatgccaagtacgccccctattgacgtcaatgacggtaaatggcccgcctggcattatgcccagtacatgaccttatgggactttcctacttggcagtacatctacgtattagtcatcgctattaccatggtcgaggtgagccccacgttctgcttcactctccccatctcccccccctccccacccccaattttgtatttatttattttttaattattttgtgcagcgatgggggcggggggggggggggggcgcgcgccaggcggggcggggcggggcgaggggcggggcggggcgaggcggagaggtgcggcggcagccaatcagagcggcgcgctccgaaagtttccttttatggcgaggcggcggcggcggcggccctataaaaagcgaagcgcgcggcgggcg

SEQ ID NO: 60 - DNA, 1182 bp, Homo sapiens
  misc_feature 1..1182: note = Strong expression promoter from human elongation factor 1 alpha
  source 1..1182: mol_type = genomic DNA
gctccggtgcccgtcagtgggcagagcgcacatcgcccacagtccccgagaagttggggggaggggtcggcaattgaaccggtgcctagagaaggtggcgcggggtaaactgggaaagtgatgtcgtgtactggctccgcctttttcccgagggtgggggagaaccgtatataagtgcagtagtcgccgtgaacgttctttttcgcaacgggtttgccgccagaacacaggtaagtgccgtgtgtggttcccgcgggcctggcctctttacgggttatggcccttgcgtgccttgaattacttccacgcccctggctgcagtacgtgattcttgatcccgagcttcgggttggaagtgggtgggagagttcgaggccttgcgcttaaggagccccttcgcctcgtgcttgagttgaggcctggcctgggcgctggggccgccgcgtgcgaatctggtggcaccttcgcgcctgtctcgctgctttcgataagtctctagccatttaaaatttttgatgacctgctgcgacgctttttttctggcaagatagtcttgtaaatgcgggccaagatctgcacactggtatttcggtttttggggccgcgggcggcgacggggcccgtgcgtcccagcgcacatgttcggcgaggcggggcctgcgagcgcggccaccgagaatcggacgggggtagtctcaagctggccggcctgctctggtgcctggcctcgcgccgccgtgtatcgccccgccctgggcggcaaggctggcccggtcggcaccagttgcgtgagcggaaagatggccgcttcccggccctgctgcagggagctcaaaatggaggacgcggcgctcgggagagcgggcgggtgagtcacccacacaaaggaaaagggcctttccgtcctcagccgtcgcttcatgtgactccacggagtaccgggcgccgtccaggcacctcgattagttctcgagcttttggagtacgtcgtctttaggttggggggaggggttttatgcgatggagtttccccacactgagtgggtggagactgaagttaggccagcttggcacttgatgtaattctccttggaatttgccctttttgagtttggatcttggttcattctcaagcctcagacagtggttcaaagtttttttcttccatttcaggtgtcgtga

SEQ ID NO: 61 - DNA, 1212 bp, Homo sapiens
  misc_feature 1..1212: note = Human B-actin
  source 1..1212: mol_type = genomic DNA
ggcctccgcgccgggttttggcgcctcccgcgggcgcccccctcctcacggcgagcgctgccacgtcagacgaagggcgcagcgagcgtcctgatccttccgcccggacgctcaggacagcggcccgctgctcataagactcggccttagaaccccagtatcagcagaaggacattttaggacgggacttgggtgactctagggcactggttttctttccagagagcggaacaggcgaggaaaagtagtcccttctcggcgattctgcggagggatctccgtggggcggtgaacgccgatgattatataaggacgcgccgggtgtggcacagctagttccgtcgcagccgggatttgggtcgcggttcttgtttgtggatcgctgtgatcgtcacttggtgagtagcgggctgctgggctggccggggctttcgtggccgccgggccgctcggtgggacggaagcgtgtggagagaccgccaagggctgtagtctgggtccgcgagcaaggttgccctgaactgggggttggggggagcgcagcaaaatggcggctgttcccgagtcttgaatggaagacgcttgtgaggcgggctgtgaggtcgttgaaacaaggtggggggcatggtgggcggcaagaacccaaggtcttgaggccttcgctaatgcgggaaagctcttattcgggtgagatgggctggggcaccatctggggaccctgacgtgaagtttgtcactgactggagaactcggtttgtcgtctgttgcgggggcggcagttatggcggtgccgttgggcagtgcacccgtacctttgggagcgcgcgccctcgtcgtgtcgtgacgtcacccgttctgttggcttataatgcagggtggggccacctgccggtaggtgtgcggtaggcttttctccgtcgcaggacgcagggttcgggcctagggtaggctctcctgaatcgacaggcgccggacctctggtgaggggagggataagtgaggcgtcagtttctttggtcggttttatgtacctatcttcttaagtagctgaagctccggttttgaactatgcgctcggggttggcgagtgtgttttgtgaagttttttaggcaccttttgaaatgtaatcatttgggtcaatatgtaattttcagtgttagactagtaaattgtccgctaaattctggccgtttttggcttttttgttagac

SEQ ID NO: 62 - DNA, 211 bp, unidentified
  misc_feature 1..211: note = NFK-b
  source 1..211: mol_type = unassigned DNA
gctagcgggaatttccgggaatttccgggaatttccgggaatttccagatctgccgccccgactgcatctgcgtgttcgaattcgccaatgacaagacgctgggcggggtttgtgtcatcatagaactaaagacatgcaaatatatttcttccggggacaccgccagcaaacgcgagcaacgggccacggggatgaagcagaagcttggca

SEQ ID NO: 63 - DNA, 1211 bp, Homo sapiens
  misc_feature 1..1211: note = Promoter of the human ubiquitin C gene (UBC)
  source 1..1211: mol_type = genomic DNA
gtctaacaaaaaagccaaaaacggccagaatttagcggacaatttactagtctaacactgaaaattacatattgacccaaatgattacatttcaaaaggtgcctaaaaaacttcacaaaacacactcgccaaccccgagcgcatagttcaaaaccggagcttcagctacttaagaagataggtacataaaaccgaccaaagaaactgacgcctcacttatccctcccctcaccagaggtccggcgcctgtcgattcaggagagcctaccctaggcccgaaccctgcgtcctgcgacggagaaaagcctaccgcacacctaccggcaggtggccccaccctgcattataagccaacagaacgggtgacgtcacgacacgacgagggcgcgcgctcccaaaggtacgggtgcactgcccaacggcaccgccataactgccgcccccgcaacagacgacaaaccgagttctccagtcagtgacaaacttcacgtcagggtccccagatggtgccccagcccatctcacccgaataagagctttcccgcattagcgaaggcctcaagaccttgggttcttgccgcccaccatgccccccaccttgtttcaacgacctcacagcccgcctcacaagcgtcttccattcaagactcgggaacagccgccattttgctgcgctccccccaacccccagttcagggcaaccttgctcgcggacccagactacagcccttggcggtctctccacacgcttccgtcccaccgagcggcccggcggccacgaaagccccggccagcccagcagcccgctactcaccaagtgacgatcacagcgatccacaaacaagaaccgcgacccaaatcccggctgcgacggaactagctgtgccacacccggcgcgtccttatataatcatcggcgttcaccgccccacggagatccctccgcagaatcgccgagaagggactacttttcctcgcctgttccgctctctggaaagaaaaccagtgccctagagtcacccaagtcccgtcctaaaatgtccttctgctgatactggggttctaaggccgagtcttatgagcagcgggccgctgtcctgagcgtccgggcggaaggatcaggacgctcgctgcgcccttcgtctgacgtggcagcgctcgccgtgaggaggggggcgcccgcgggaggcgccaaaacccggcgcggaggc

SEQ ID NO: 64 - DNA, 317 bp, synthetic construct
  misc_feature 1..317: note = Synthetic: Mammalian expression promoter from the simian vacuolating virus 40
  source 1..317: mol_type = other DNA
ggtgtggaaagtccccaggctccccagcaggcagaagtatgcaaagcatgcatctcaattagtcagcaaccaggtgtggaaagtccccaggctccccagcaggcagaagtatgcaaagcatgcatctcaattagtcagcaaccatagtcccgcccctaactccgcccatcccgcccctaactccgcccagttccgcccattctccgccccatggctgactaattttttttatttatgcagaggccgaggccgcctcggcctctgagctattccagaagtagtgaggaggcttttttggaggcctaggcttttgcaaa

SEQ ID NO: 65 - DNA, 399 bp, unidentified
  misc_feature 1..399: note = Promoter from human or mouse phosphoglycerate kinase gene (PGK)
  source 1..399: mol_type = unassigned DNA
ccggtaggcgccaaccggctccgttctttggtggccccttcgcgccaccttctactcctcccctagtcaggaagttcccccccgccccgcagctcgcgtcgtgcaggacgtgacaaatggaagtagcacgtctcactagtctcgtgcagatggacagcaccgctgagcaatggaagcgggtaggcctttggggcagcggccaatagcagctttgctccttcgctttctgggctcagaggctgggaaggggtgggtccgggggcgggctcaggggcgggctcaggggcggggcgggcgcccgaaggtcctccggaggcccggcattctgcacgcttcaaaagcgcacgtctgccgcgctgttctcctcttcctcatctccgggcctttcgacctgcagcc

SEQ ID NO: 66 - DNA, 99 bp, Homo sapiens
  misc_feature 1..99: note = Promoter from the human polymerase III RNA promoter
  source 1..99: mol_type = genomic DNA
aatatttgcatgtcgctatgtgttctgggaaatcaccataaacgtgaaatgtctttggatttgggaatcttataagttctgtatgagaccacagatccc

SEQ ID NO: 67 - DNA, 314 bp, Homo sapiens
  misc_feature 1..314: note = Promoter from the human U6 small nuclear promoter
  source 1..314: mol_type = genomic DNA
gatccgacgccgccatctctaggcccgcgccggccccctcgcacagacttgtgggagaagctcggctactcccctgccccggttaatttgcatataatatttcctagtaactatagaggcttaatgtgcgataaaagacagataatctgttctttttaatactagctacattttacatgataggcttggatttctataagagatacaaatactaaattattattttaaaaaacagcacaaaaggaaactcaccctaactgtaaagtaattgtgtgttttgagactataaatatcccttggagaaaagccttgtt

SEQ ID NO: 68 - DNA, 250 bp, synthetic construct
  misc_feature 1..250: note = Synthetic: 250 bp S/MAR
  source 1..250: mol_type = other DNA
tctttaatttctaatatatttagaatctttaatttctaatatatttagaatctttaatttctaatatatttagaatctttaatttctaatatatttagaatctttaatttctaatatatttagaatctttaatttctaatatatttagaatctttaatttctaatatatttagaatctttaatttctaatatatttagaatctttaatttctaatatatttagaatctttaatttctaatatatttagaa

SEQ ID NO: 69 - DNA, 250 bp, synthetic construct; identical to SEQ ID NO: 68
  misc_feature 1..250: note = Synthetic: 439 bp S/MAR
  source 1..250: mol_type = other DNA

SEQ ID NO: 70 - DNA, 45 bp, synthetic construct
  misc_feature 1..45: note = Synthetic: (45 bp) Type A
  source 1..45: mol_type = other DNA
ggtgcatcgatgcagcatcgaggcaggtgcatcgatacagggggg

SEQ ID NO: 71 - DNA, 24 bp, synthetic construct
  misc_feature 1..24: note = Synthetic: (24 bp) Type B
  source 1..24: mol_type = other DNA
tcgtcgttttgtcgttttgtcgtt

SEQ ID NO: 72 - DNA, 21 bp, synthetic construct
  misc_feature 1..21: note = Synthetic: (21 bp) Type C
  source 1..21: mol_type = other DNA
tcgtcgaacgttcgagatgat

SEQ ID NO: 73 - DNA, 130 bp, synthetic construct
  misc_feature 1..130: note = Synthetic: B-globin intron
  source 1..130: mol_type = other DNA
gttggtatcaaggttacaagacaggtttaaggagaccaatagaaactgggcatgtggagacagagaagactcttgggtttctgataggcactgactctctctgcctattggtctattttcccacccttag

SEQ ID NO: 74 - DNA, 262 bp, Homo sapiens
  misc_feature 1..262: note = Human growth hormone intron
  source 1..262: mol_type = genomic DNA
ttcgaacaggtaagcgcccctaaaatccctttgggcacaatgtgtcctgaggggagaggcagcgacctgtagatgggacgggggcactaaccctcaggtttggggcttctgaatgtgagtatcgccatgtaagcccagtatttggccaatctcagaaagctcctggtccctggagggatggagagagaaaaacaaacagctcctggagcagggagagtgctggcctcttgctctccggctccctctgttgccctctggtttc

SEQ ID NO: 75 - protein, 15 aa, synthetic construct
  REGION 1..15: note = Synthetic: peptide
SSSPVSPADDSGSNS

SEQ ID NO: 76 - protein, 9 aa, synthetic construct
  REGION 1..9: note = Synthetic: peptide
SKENQSENS

SEQ ID NO: 77 - protein, 11 aa, synthetic construct
  REGION 1..11: note = Synthetic: peptide
SKENIMRSENS

SEQ ID NO: 78 - protein, 9 aa, synthetic construct
  REGION 1..9: note = Synthetic: peptide
RTALGDIGN

SEQ ID NO: 79 - protein, 9 aa, synthetic construct
  REGION 1..9: note = Synthetic: peptide
RNMLANAEN

SEQ ID NO: 80 - protein, 9 aa, synthetic construct
  REGION 1..9: note = Synthetic: peptide
RAALAVLKS

SEQ ID NO: 81 - DNA, 1800 bp, synthetic construct
  misc_feature 1..1800: note = Synthetic: cDNA Sequence
  source 1..1800: mol_type = other DNA
atggggctgctgtcccagggctcgccgctgagctgggaggaaaccaagcgccatgccgaccacgtgcggcggcacgggatcctccagttcctgcacatctaccacgccgtcaaggaccggcacaaggacgttctcaagtggggcgatgaggtggaatacatgttggtatcttttgatcatgaaaataaaaaagtccggttggtcctgtctggggagaaagttcttgaaactctgcaagagaagggggaaaggacaaacccaaaccatcctaccctttggagaccagagtatgggagttacatgattgaagggacaccaggacagccctacggaggaacaatgtccgagttcaatacagttgaggccaacatgcgaaaacgccggaaggaggctacttctatattagaagaaaatcaggctctttgcacaataacttcatttcccagtaccttaacaagaaatatccgacataggagaggagaaaaggttgtcatcaatgtaccaatatttaaggacaagaatacaccatctccatttatagaaacatttactgaggatgatgaagcttcaagggcttctaagccggatcatatttacatggatgccatgggatttggaatgggcaattgctgtctccaggtgacattccaagcctgcagtatatctgaggccagatacctttatgatcagttggctactatctgtccaattgttatggctttgagtgctgcatctcccttttaccgaggctatgtgtcagacattgattgtcgctggggagtgatttctgcatctgtagatgatagaactcgggaggagcgaggactggagccattgaagaacaataactataggatcagtaaatcccgatatgactcaatagacagctatttatctaagtgtggtgagaaatataatgacatcgacttgacgatagataaagagatctacgaacagctgttgcaggaaggcattgatcatctcctggcccagcatgttgctcatctctttattagagacccactgacactgtttgaagagaaaatacacctggatgatgctaatgagtctgaccattttgagaatattcagtccacaaattggcagacaatgagatttaagccccctcctccaaactcagacattggatggagagtagaatttcgacccatggaggtgcaattaacagactttgagaactctgcctatgtggtgtttgtggtactgctcaccagagtgatcctttcctacaaattggattttctcattccactgtcaaaggttgatgagaacatgaaggtagcacagaaaagagatgctgtcttgcagggaatgttttatttcaggaaagatatttgcaaaggtggcaatgcagtggtggatggttgtggcaaggcccagaacagcacggagctcgctgcagaggagtacaccctcatgagcatagacaccatcatcaatgggaaggaaggtgtgtttcctggactgatcccaattctgaactcttaccttgaaaacatggaagtggatgtggacaccagatgtagtattctgaactacctaaagctaattaagaagagagcatctggagaactaatgacagttgccagatggatgagggagtttatcgcaaaccatcctgactacaagcaagacagtgtcataactgatgaaatgaattatagccttattttgaagtgtaaccaaattgcaaatgaattatgtgaatgcccagagttacttggatcagcatttaggaaagtaaaatatagtggaagtaaaactgactcatccaactag

SEQ ID NO: 82 - DNA, 759 bp, synthetic construct
  misc_feature 1..759: note = Synthetic: cDNA Sequence
  source 1..759: mol_type = other DNA
atgggcaccgacagccgcgcggccaaggcgctcctggcgcgggcccgcaccctgcacctgcagacggggaacctgctgaactggggccgcctgcggaagaagtgcccgtccacgcacagcgaggaggagtttccagatgtcttggaatgcactgtatctcatgcagtagaaaagataaatcctgatgaaagagaagaaatgaaagtttctgcaaaactgttcattgtagaatcaaactcttcatcatcaactagaagtgcagttgacatggcctgttcagtccttggagttgcacagctggattctgtgatcattgcttcacctcctattgaagatggagttaatctttccttggagcatttacagccttactgggaggaattagaaaacttagttcagagcaaaaagattgttgccataggtacctctgatctagacaaaacacagttggaacagctgtatcagtgggcacaggtaaaaccaaatagtaaccaagttaatcttgcctcctgctgtgtgatgccaccagatttgactgcatttgctaaacaatttgacatacagctgttgactcacaatgatccaaaagaactgctttctgaagcaagtttccaagaagctcttcaggaaagcattcctgacattcaagcgcacgagtgggtgccgctgtggctactgcggtattcggtcattgtgaaaagtagaggaattatcaaatcaaaaggctacattttacaagctaaaagaaggggttcttaa

SEQ ID NO: 83 - DNA, 1569 bp, synthetic construct
  misc_feature 1..1569: note = Synthetic: cDNA Sequence
  source 1..1569: mol_type = other DNA
atggccctgctgccccgagccctgagcgccggcgcgggaccgagctggcggcgggcggcgcgcgccttccgaggcttcctgctgcttctgcccgagcccgcggccctcacgcgcgccctctcccgtgccatggcctgcaggcaggagccgcagccgcagggcccgccgcccgctgctggcgccgtggcctcctatgactacctggtgatcgggggcggctcgggcgggctggccagcgcgcgcagggcggccgagctgggtgccagggccgccgtggtggagagccacaagctgggtggcacttgcgtgaatgttggatgtgtacccaaaaaggtaatgtggaacacagctgtccactctgaattcatgcatgatcatgctgattatggctttccaagttgtgagggtaaattcaattggcgtgttattaaggaaaagcgggatgcctatgtgagccgcctgaatgccatctatcaaaacaatctcaccaagtcccatatagaaatcatccgtggccatgcagccttcacgagtgatcccaagcccacaatagaggtcagtgggaaaaagtacaccgccccacacatcctgatcgccacaggtggtatgccctccacccctcatgagagccagatccccggtgccagcttaggaataaccagcgatggattttttcagctggaagaattgcccggccgcagcgtcattgttggtgcaggttacattgctgtggagatggcagggatcctgtcagccctgggttctaagacatcactgatgatacggcatgataaggtacttagaagttttgattcaatgatcagcaccaactgcacggaggagctggagaacgctggcgtggaggtgctgaagttctcccaggtcaaggaggttaaaaagactttgtcgggcttggaagtcagcatggttactgcagttcccggtaggctaccagtcatgaccatgattccagatgttgactgcctgctctgggccattgggcgggtcccgaataccaaggacctgagtttaaacaaactggggattcaaaccgatgacaagggtcatatcatcgtagacgaattccagaataccaacgtcaaaggcatctatgcagttggggatgtatgtggaaaagctcttcttactccagttgcaatagctgctggccgaaaacttgcccatcgactttttgaatataaggaagattccaaattagattataacaacatcccaactgtggtcttcagccacccccctattgggacagtgggactcacggaagatgaagccattcataaatatggaatagaaaatgtgaagacctattcaacgagctttaccccgatgtatcacgcagttaccaaaaggaaaacaaaatgtgtgatgaaaatggtctgtgctaacaaggaagaaaaggtggttgggatccatatgcagggacttgggtgtgatgaaatgctgcagggttttgctgttgcagtgaagatgggagcaacgaaggcagactttgacaacacagtcgccattcaccctacctcttcagaagagctggtcacacttcgttga

SEQ ID NO: 84 - DNA, 558 bp, Homo sapiens
  misc_feature 1..558: note = RLN2 (human)
  source 1..558: mol_type = genomic DNA
atgcctcgcctgttttttttccacctgctaggagtctgtttactactgaaccaattttccagagcagtcgcggactcatggatggaggaagttattaaattatgcggccgcgaattagttcgcgcgcagattgccatttgcggcatgagcacctggagcaaaaggtctctgagccaggaagatgctcctcagacacctagaccagtggcagaaattgtgccatccttcatcaacaaagatacagaaaccataaatatgatgtcagaatttgttgctaatttgccacaggagctgaagttaaccctgtctgagatgcagccagcattaccacagctacaacaacatgtacctgtattaaaagattccagtcttctctttgaagaatttaagaaacttattcgcaatagacaaagtgaagccgcagacagcagtccttcagaattaaaatacttaggcttggatactcattctcgaaaaaagagacaactctacagtgcattggctaataaatgttgccatgttggttgtaccaaaagatctcttgctagattttgctga

SEQ ID NO: 85 - DNA, 555 bp, Mus musculus
  misc_feature 1..555: note = RLN1 (mouse)
  source 1..555: mol_type = genomic DNA
atgtccagcagatttttgctccagctcctggggttctggctattgctgagccagccttgcaggacgcgagtctcggaggagtggatggacggattcattcggatgtgcggccgtgaatatgcccgtgaattgatcaaaatctgcggggcctccgtgggaagattggctttgagccaggaggagccagctctgcttgccaggcaagccactgaagttgtgccatccttcatcaacaaagatgcagagcctttcgatacgacgctgaaatgccttccaaatttgtctgaagagctcaaggcagtactgtctgaggctcaggcctcgctcccagagctacaacacgcacctgtgttgagcgattctgttgttagcttggaaggctttaagaaaactctccatgataaactgggtgaagcagaagacggcagtcctccagggcttaaatacttgcaatcagatacccattcacggaaaaagagggagtctggtggattgatgagccagcaatgttgccacgtcggttgtagcagaagatctattgctaaactctattgc

SEQ ID NO: 86 - DNA, 55 bp, unidentified
  misc_feature 1..55: note = Binding site of nuclear factor kappa-light-chain-enhancer of activated B cells
  source 1..55: mol_type = unassigned DNA
ggggactttccggggactttccggggactttccggggactttccggggactttcc

SEQ ID NO: 87 - DNA, 20 bp, unidentified
  misc_feature 1..20: note = Binding site of tumor protein 53 (p53)
  source 1..20: mol_type = unassigned DNA
agactgggcatgtctgggca

SEQ ID NO: 88 - DNA, 20 bp, unidentified
  misc_feature 1..20: note = Binding site of tumor protein 53 (p53)
  source 1..20: mol_type = unassigned DNA
gaacatgtcccaacatgttg

SEQ ID NO: 89 - DNA, 15 bp, unidentified
  misc_feature 1..15: note = Adenovirus major late promoter
  source 1..15: mol_type = unassigned DNA
ggggctataaaaggg